European Patent Specification EP 3 897 696 B1, published August 20, 2025. Title: EXTRACORPOREAL DEVICES AND METHODS FOR TREATING DISEASES ASSOCIATED WITH ANTI-NEUTROPHIL CYTOPLASMIC ANTIBODIES. Applicant: Gambro Lundia AB. The sequence listing filed with the application follows.

SEQUENCE LISTING (7 sequences)

SEQ ID NO: 1 - protein, 256 aa, Homo sapiens
MAHRPPSPALASVLLALLLSGAARAAEIVGGHEAQPHSRPYMASLQMRGNPGSHFCGGTLIHPSFVLTAAHCLRDIPQRLVNVVLGAHNVRTQEPTQQHFSVAQVFLNNYDAENKLNDVLLIQLSSPANLSASVATVQLPQQDQPVPHGTQCLAMGWGRVGAHDPPAQVLQELNVTVVTFFCRPHNICTFVPRRKAGICFGDSGGPLICDGIIQGIDSFVIWGCATRLFPDFFTRVALYVDWIRSTLRRVEAKGRP

SEQ ID NO: 2 - protein, 256 aa, Artificial Sequence
  variant
  misc_feature (221)..(221): Xaa can be any naturally occurring amino acid
MAHRPPSPALASVLLALLLSGAARAAEIVGGHEAQPHSRPYMASLQMRGNPGSHFCGGTLIHPSFVLTAAHCLRDIPQRLVNVVLGAHNVRTQEPTQQHFSVAQVFLNNYDAENKLNDVLLIQLSSPANLSASVATVQLPQQDQPVPHGTQCLAMGWGRVGAHDPPAQVLQELNVTVVTFFCRPHNICTFVPRRKAGICFGDSGGPLICDGIIQGIDSFVXWGCATRLFPDFFTRVALYVDWIRSTLRRVEAKGRP

SEQ ID NO: 3 - protein, 256 aa, Artificial Sequence
  variant
  misc_feature (221)..(222): Xaa can be any naturally occurring amino acid
MAHRPPSPALASVLLALLLSGAARAAEIVGGHEAQPHSRPYMASLQMRGNPGSHFCGGTLIHPSFVLTAAHCLRDIPQRLVNVVLGAHNVRTQEPTQQHFSVAQVFLNNYDAENKLNDVLLIQLSSPANLSASVATVQLPQQDQPVPHGTQCLAMGWGRVGAHDPPAQVLQELNVTVVTFFCRPHNICTFVPRRKAGICFGDSGGPLICDGIIQGIDSFVXXGCATRLFPDFFTRVALYVDWIRSTLRRVEAKGRP

SEQ ID NO: 4 - protein, 256 aa, Artificial Sequence
  variant
  misc_feature (71)..(71): Xaa can be any naturally occurring amino acid
  misc_feature (118)..(118): Xaa can be any naturally occurring amino acid
  misc_feature (203)..(203): Xaa can be any naturally occurring amino acid
  misc_feature (221)..(221): Xaa can be any naturally occurring amino acid
MAHRPPSPALASVLLALLLSGAARAAEIVGGHEAQPHSRPYMASLQMRGNPGSHFCGGTLIHPSFVLTAAXCLRDIPQRLVNVVLGAHNVRTQEPTQQHFSVAQVFLNNYDAENKLNXVLLIQLSSPANLSASVATVQLPQQDQPVPHGTQCLAMGWGRVGAHDPPAQVLQELNVTVVTFFCRPHNICTFVPRRKAGICFGDXGGPLICDGIIQGIDSFVXWGCATRLFPDFFTRVALYVDWIRSTLRRVEAKGRP

SEQ ID NO: 5 - protein, 256 aa, Artificial Sequence
  variant
  misc_feature (71)..(71): Xaa can be any naturally occurring amino acid
  misc_feature (118)..(118): Xaa can be any naturally occurring amino acid
  misc_feature (203)..(203): Xaa can be any naturally occurring amino acid
  misc_feature (221)..(222): Xaa can be any naturally occurring amino acid
MAHRPPSPALASVLLALLLSGAARAAEIVGGHEAQPHSRPYMASLQMRGNPGSHFCGGTLIHPSFVLTAAXCLRDIPQRLVNVVLGAHNVRTQEPTQQHFSVAQVFLNNYDAENKLNXVLLIQLSSPANLSASVATVQLPQQDQPVPHGTQCLAMGWGRVGAHDPPAQVLQELNVTVVTFFCRPHNICTFVPRRKAGICFGDXGGPLICDGIIQGIDSFVXXGCATRLFPDFFTRVALYVDWIRSTLRRVEAKGRP

SEQ ID NO: 6 - protein, 256 aa, Artificial Sequence
  variant
MAHRPPSPALASVLLALLLSGAARAAEIVGGHEAQPHSRPYMASLQMRGNPGSHFCGGTLIHPSFVLTAAHCLRDIPQRLVNVVLGAHNVRTQEPTQQHFSVAQVFLNNYDAENKLNDVLLIQLSSPANLSASVATVQLPQQDQPVPHGTQCLAMGWGRVGAHDPPAQVLQELNVTVVTFFCRPHNICTFVPRRKAGICFGDAGGPLICDGIIQGIDSFVAWGCATRLFPDFFTRVALYVDWIRSTLRRVEAKGRP

SEQ ID NO: 7 - protein, 256 aa, Artificial Sequence
  variant
MAHRPPSPALASVLLALLLSGAARAAEIVGGHEAQPHSRPYMASLQMRGNPGSHFCGGTLIHPSFVLTAAHCLRDIPQRLVNVVLGAHNVRTQEPTQQHFSVAQVFLNNYDAENKLNDVLLIQLSSPANLSASVATVQLPQQDQPVPHGTQCLAMGWGRVGAHDPPAQVLQELNVTVVTFFCRPHNICTFVPRRKAGICFGDAGGPLICDGIIQGIDSFVAAGCATRLFPDFFTRVALYVDWIRSTLRRVEAKGRP